European Patent Specification EP 3 835 311 B1, published August 28, 2024. Title: Nkx3.2 FRAGMENT AND PHARMACEUTICAL COMPOSITION COMPRISING SAME AS ACTIVE INGREDIENT. Applicant: ICM Co., Ltd. The sequence listing filed with the application follows.

SEQUENCE LISTING (42 sequences)

SEQ ID NO: 1 - protein, 144 aa, Artificial Sequence
  166-309 aa fragment of Nkx3.2
GVGPRGAHVSALCSGAGGGGGSGPAGVAEEEEEPAAPKPRKKRSRAAFSHAQVFELERRFNHQRYLSGPERADLAASLKLTETQVKIWFQNRRYKTKRRQMAADLLASAPAAKKVAVKVLVRDDQRQYLPGEVLRPPSLLPLQP

SEQ ID NO: 2 - DNA, 432 bp, Artificial Sequence
  nucleotide sequence encoding 166-309 aa fragment of Nkx3.2
ggtgttggccccagaggtgcacacgtgtccgcgctgtgcagcggggccggcggcgggggcggcagcgggccggcaggcgtcgcggaggaggaggaggagccggcggcgcccaagccacgcaagaagcgctcgcgggccgctttctcccacgcgcaggtcttcgagctggagcgccgctttaaccaccagcgctacctgtccgggcccgagcgcgcagacctggccgcgtcgctgaagctcaccgagacgcaggtgaaaatctggttccagaaccgtcgctacaagacaaagcgccggcagatggcagccgacctgctggcctcggcgcccgccgccaagaaggtggccgtaaaggtgctggtgcgcgacgaccagagacaatacctgcccggcgaagtgctgcggccaccctcgcttctgccactgcagccc

SEQ ID NO: 3 - protein, 43 aa, Artificial Sequence
  123-165 aa fragment of Nkx3.2
LSLGQPVCELAASKDLEEEAAGRSDSEMSASVSGDRSPRTEDD

SEQ ID NO: 4 - DNA, 129 bp, Artificial Sequence
  nucleotide sequence encoding 123-165 aa fragment of Nkx3.2
ttgagcctcggccagccggtctgtgagctggccgcttccaaagacctagaggaggaagccgcgggccggagcgacagcgagatgtccgccagcgtctcaggcgaccgcagcccaaggaccgaggacgac

SEQ ID NO: 5 - protein, 24 aa, Artificial Sequence
  310-333 aa fragment encoding Nkx3.2
SYYYPYYCLPGWALSTCAAAAGTQ

SEQ ID NO: 6 - DNA, 72 bp, Artificial Sequence
  nucleotide sequence encoding 310-333 aa fragment of Nkx3.2
tcctactattacccgtactactgcctcccaggctgggcgctctccacctgcgcagctgccgcaggcacccag

SEQ ID NO: 7 - protein, 333 aa, Homo sapiens
MAVRGANTLTSFSIQAILNKKEERGGLAAPEGRPAPGGTAASVAAAPAVCCWRLFGERDAGALGGAEDSLLASPAGTRTAAGRTAESPEGWDSDSALSEENESRRRCADARGASGAGLAGGSLSLGQPVCELAASKDLEEEAAGRSDSEMSASVSGDRSPRTEDDGVGPRGAHVSALCSGAGGGGGSGPAGVAEEEEEPAAPKPRKKRSRAAFSHAQVFELERRFNHQRYLSGPERADLAASLKLTETQVKIWFQNRRYKTKRRQMAADLLASAPAAKKVAVKVLVRDDQRQYLPGEVLRPPSLLPLQPSYYYPYYCLPGWALSTCAAAAGTQ

SEQ ID NO: 8 - DNA, 1002 bp, Homo sapiens
atggctgtgcgcggcgccaacaccttgacgtccttctccatccaggcgatcctcaacaagaaagaggagcgcggcgggctggccgcgccagaggggcgcccggcgcccgggggcacagcggcatcggtggccgcggctcccgctgtctgctgttggcggctctttggggagagggacgcgggcgcgttggggggcgccgaggactctctgctggcgtctcctgccggtaccagaacagctgcggggcggactgcggagagcccggaaggctgggactcggactccgcgctcagcgaggagaacgagagcaggcggcgctgcgcggacgcgcggggggccagcggggccggccttgcggggggatccttgagcctcggccagccggtctgtgagctggccgcttccaaagacctagaggaggaagccgcgggccggagcgacagcgagatgtccgccagcgtctcaggcgaccgcagcccaaggaccgaggacgacggtgttggccccagaggtgcacacgtgtccgcgctgtgcagcggggccggcggcgggggcggcagcgggccggcaggcgtcgcggaggaggaggaggagccggcggcgcccaagccacgcaagaagcgctcgcgggccgctttctcccacgcgcaggtcttcgagctggagcgccgctttaaccaccagcgctacctgtccgggcccgagcgcgcagacctggccgcgtcgctgaagctcaccgagacgcaggtgaaaatctggttccagaaccgtcgctacaagacaaagcgccggcagatggcagccgacctgctggcctcggcgcccgccgccaagaaggtggccgtaaaggtgctggtgcgcgacgaccagagacaatacctgcccggcgaagtgctgcggccaccctcgcttctgccactgcagccctcctactattacccgtactactgcctcccaggctgggcgctctccacctgcgcagctgccgcaggcacccagtga

SEQ ID NO: 9 - protein, 320 aa, Artificial Sequence
  1-320 aa fragment of Nkx3.2
MAVRGANTLTSFSIQAILNKKEERGGLAAPEGRPAPGGTAASVAAAPAVCCWRLFGERDAGALGGAEDSLLASPAGTRTAAGRTAESPEGWDSDSALSEENESRRRCADARGASGAGLAGGSLSLGQPVCELAASKDLEEEAAGRSDSEMSASVSGDRSPRTEDDGVGPRGAHVSALCSGAGGGGGSGPAGVAEEEEEPAAPKPRKKRSRAAFSHAQVFELERRFNHQRYLSGPERADLAASLKLTETQVKIWFQNRRYKTKRRQMAADLLASAPAAKKVAVKVLVRDDQRQYLPGEVLRPPSLLPLQPSYYYPYYCLPG

SEQ ID NO: 10 - protein, 307 aa, Artificial Sequence
  1-307 aa fragment of Nkx3.2
MAVRGANTLTSFSIQAILNKKEERGGLAAPEGRPAPGGTAASVAAAPAVCCWRLFGERDAGALGGAEDSLLASPAGTRTAAGRTAESPEGWDSDSALSEENESRRRCADARGASGAGLAGGSLSLGQPVCELAASKDLEEEAAGRSDSEMSASVSGDRSPRTEDDGVGPRGAHVSALCSGAGGGGGSGPAGVAEEEEEPAAPKPRKKRSRAAFSHAQVFELERRFNHQRYLSGPERADLAASLKLTETQVKIWFQNRRYKTKRRQMAADLLASAPAAKKVAVKVLVRDDQRQYLPGEVLRPPSLLPL

SEQ ID NO: 11 - protein, 292 aa, Artificial Sequence
  42-333 aa fragment of Nkx3.2
SVAAAPAVCCWRLFGERDAGALGGAEDSLLASPAGTRTAAGRTAESPEGWDSDSALSEENESRRRCADARGASGAGLAGGSLSLGQPVCELAASKDLEEEAAGRSDSEMSASVSGDRSPRTEDDGVGPRGAHVSALCSGAGGGGGSGPAGVAEEEEEPAAPKPRKKRSRAAFSHAQVFELERRFNHQRYLSGPERADLAASLKLTETQVKIWFQNRRYKTKRRQMAADLLASAPAAKKVAVKVLVRDDQRQYLPGEVLRPPSLLPLQPSYYYPYYCLPGWALSTCAAAAGTQ

SEQ ID NO: 12 - protein, 235 aa, Artificial Sequence
  99-333 aa fragment of Nkx3.2
EENESRRRCADARGASGAGLAGGSLSLGQPVCELAASKDLEEEAAGRSDSEMSASVSGDRSPRTEDDGVGPRGAHVSALCSGAGGGGGSGPAGVAEEEEEPAAPKPRKKRSRAAFSHAQVFELERRFNHQRYLSGPERADLAASLKLTETQVKIWFQNRRYKTKRRQMAADLLASAPAAKKVAVKVLVRDDQRQYLPGEVLRPPSLLPLQPSYYYPYYCLPGWALSTCAAAAGTQ

SEQ ID NO: 13 - protein, 222 aa, Artificial Sequence
  112-333 aa fragment of Nkx3.2
GASGAGLAGGSLSLGQPVCELAASKDLEEEAAGRSDSEMSASVSGDRSPRTEDDGVGPRGAHVSALCSGAGGGGGSGPAGVAEEEEEPAAPKPRKKRSRAAFSHAQVFELERRFNHQRYLSGPERADLAASLKLTETQVKIWFQNRRYKTKRRQMAADLLASAPAAKKVAVKVLVRDDQRQYLPGEVLRPPSLLPLQPSYYYPYYCLPGWALSTCAAAAGTQ

SEQ ID NO: 14 - protein, 211 aa, Artificial Sequence
  123-333 aa fragment of Nkx3.2
LSLGQPVCELAASKDLEEEAAGRSDSEMSASVSGDRSPRTEDDGVGPRGAHVSALCSGAGGGGGSGPAGVAEEEEEPAAPKPRKKRSRAAFSHAQVFELERRFNHQRYLSGPERADLAASLKLTETQVKIWFQNRRYKTKRRQMAADLLASAPAAKKVAVKVLVRDDQRQYLPGEVLRPPSLLPLQPSYYYPYYCLPGWALSTCAAAAGTQ

SEQ ID NO: 15 - protein, 232 aa, Artificial Sequence
  99-330 aa fragment of Nkx3.2
EENESRRRCADARGASGAGLAGGSLSLGQPVCELAASKDLEEEAAGRSDSEMSASVSGDRSPRTEDDGVGPRGAHVSALCSGAGGGGGSGPAGVAEEEEEPAAPKPRKKRSRAAFSHAQVFELERRFNHQRYLSGPERADLAASLKLTETQVKIWFQNRRYKTKRRQMAADLLASAPAAKKVAVKVLVRDDQRQYLPGEVLRPPSLLPLQPSYYYPYYCLPGWALSTCAAAA

SEQ ID NO: 16 - protein, 229 aa, Artificial Sequence
  99-327 aa fragment of Nkx3.2
EENESRRRCADARGASGAGLAGGSLSLGQPVCELAASKDLEEEAAGRSDSEMSASVSGDRSPRTEDDGVGPRGAHVSALCSGAGGGGGSGPAGVAEEEEEPAAPKPRKKRSRAAFSHAQVFELERRFNHQRYLSGPERADLAASLKLTETQVKIWFQNRRYKTKRRQMAADLLASAPAAKKVAVKVLVRDDQRQYLPGEVLRPPSLLPLQPSYYYPYYCLPGWALSTCA

SEQ ID NO: 17 - protein, 222 aa, Artificial Sequence
  99-320 aa fragment of Nkx3.2
EENESRRRCADARGASGAGLAGGSLSLGQPVCELAASKDLEEEAAGRSDSEMSASVSGDRSPRTEDDGVGPRGAHVSALCSGAGGGGGSGPAGVAEEEEEPAAPKPRKKRSRAAFSHAQVFELERRFNHQRYLSGPERADLAASLKLTETQVKIWFQNRRYKTKRRQMAADLLASAPAAKKVAVKVLVRDDQRQYLPGEVLRPPSLLPLQPSYYYPYYCLPG

SEQ ID NO: 18 - protein, 223 aa, Artificial Sequence
  105-327 aa fragment of Nkx3.2
RRCADARGASGAGLAGGSLSLGQPVCELAASKDLEEEAAGRSDSEMSASVSGDRSPRTEDDGVGPRGAHVSALCSGAGGGGGSGPAGVAEEEEEPAAPKPRKKRSRAAFSHAQVFELERRFNHQRYLSGPERADLAASLKLTETQVKIWFQNRRYKTKRRQMAADLLASAPAAKKVAVKVLVRDDQRQYLPGEVLRPPSLLPLQPSYYYPYYCLPGWALSTCA

SEQ ID NO: 19 - protein, 215 aa, Artificial Sequence
  110-324 aa fragment of Nkx3.2
ARGASGAGLAGGSLSLGQPVCELAASKDLEEEAAGRSDSEMSASVSGDRSPRTEDDGVGPRGAHVSALCSGAGGGGGSGPAGVAEEEEEPAAPKPRKKRSRAAFSHAQVFELERRFNHQRYLSGPERADLAASLKLTETQVKIWFQNRRYKTKRRQMAADLLASAPAAKKVAVKVLVRDDQRQYLPGEVLRPPSLLPLQPSYYYPYYCLPGWALS

SEQ ID NO: 20 - protein, 209 aa, Artificial Sequence
  112-320 aa fragment of Nkx3.2
GASGAGLAGGSLSLGQPVCELAASKDLEEEAAGRSDSEMSASVSGDRSPRTEDDGVGPRGAHVSALCSGAGGGGGSGPAGVAEEEEEPAAPKPRKKRSRAAFSHAQVFELERRFNHQRYLSGPERADLAASLKLTETQVKIWFQNRRYKTKRRQMAADLLASAPAAKKVAVKVLVRDDQRQYLPGEVLRPPSLLPLQPSYYYPYYCLPG

SEQ ID NO: 21 - protein, 198 aa, Artificial Sequence
  123-320 aa fragment of Nkx3.2
LSLGQPVCELAASKDLEEEAAGRSDSEMSASVSGDRSPRTEDDGVGPRGAHVSALCSGAGGGGGSGPAGVAEEEEEPAAPKPRKKRSRAAFSHAQVFELERRFNHQRYLSGPERADLAASLKLTETQVKIWFQNRRYKTKRRQMAADLLASAPAAKKVAVKVLVRDDQRQYLPGEVLRPPSLLPLQPSYYYPYYCLPG

SEQ ID NO: 22 - protein, 191 aa, Artificial Sequence
  130-320 aa fragment of Nkx3.2
CELAASKDLEEEAAGRSDSEMSASVSGDRSPRTEDDGVGPRGAHVSALCSGAGGGGGSGPAGVAEEEEEPAAPKPRKKRSRAAFSHAQVFELERRFNHQRYLSGPERADLAASLKLTETQVKIWFQNRRYKTKRRQMAADLLASAPAAKKVAVKVLVRDDQRQYLPGEVLRPPSLLPLQPSYYYPYYCLPG

SEQ ID NO: 23 - protein, 171 aa, Artificial Sequence
  150-320 aa fragment of Nkx3.2
MSASVSGDRSPRTEDDGVGPRGAHVSALCSGAGGGGGSGPAGVAEEEEEPAAPKPRKKRSRAAFSHAQVFELERRFNHQRYLSGPERADLAASLKLTETQVKIWFQNRRYKTKRRQMAADLLASAPAAKKVAVKVLVRDDQRQYLPGEVLRPPSLLPLQPSYYYPYYCLPG

SEQ ID NO: 24 - protein, 166 aa, Artificial Sequence
  153-318 aa fragment of Nkx3.2
SVSGDRSPRTEDDGVGPRGAHVSALCSGAGGGGGSGPAGVAEEEEEPAAPKPRKKRSRAAFSHAQVFELERRFNHQRYLSGPERADLAASLKLTETQVKIWFQNRRYKTKRRQMAADLLASAPAAKKVAVKVLVRDDQRQYLPGEVLRPPSLLPLQPSYYYPYYCL

SEQ ID NO: 25 - protein, 161 aa, Artificial Sequence
  156-316 aa fragment of Nkx3.2
GDRSPRTEDDGVGPRGAHVSALCSGAGGGGGSGPAGVAEEEEEPAAPKPRKKRSRAAFSHAQVFELERRFNHQRYLSGPERADLAASLKLTETQVKIWFQNRRYKTKRRQMAADLLASAPAAKKVAVKVLVRDDQRQYLPGEVLRPPSLLPLQPSYYYPYY

SEQ ID NO: 26 - protein, 156 aa, Artificial Sequence
  159-314 aa fragment of Nkx3.2
SPRTEDDGVGPRGAHVSALCSGAGGGGGSGPAGVAEEEEEPAAPKPRKKRSRAAFSHAQVFELERRFNHQRYLSGPERADLAASLKLTETQVKIWFQNRRYKTKRRQMAADLLASAPAAKKVAVKVLVRDDQRQYLPGEVLRPPSLLPLQPSYYYP

SEQ ID NO: 27 - protein, 151 aa, Artificial Sequence
  162-312 polypeptide fragment of Nkx3.2
TEDDGVGPRGAHVSALCSGAGGGGGSGPAGVAEEEEEPAAPKPRKKRSRAAFSHAQVFELERRFNHQRYLSGPERADLAASLKLTETQVKIWFQNRRYKTKRRQMAADLLASAPAAKKVAVKVLVRDDQRQYLPGEVLRPPSLLPLQPSYY

SEQ ID NO: 28 - protein, 146 aa, Artificial Sequence
  165-310 polypeptide fragment of Nkx3.2
DGVGPRGAHVSALCSGAGGGGGSGPAGVAEEEEEPAAPKPRKKRSRAAFSHAQVFELERRFNHQRYLSGPERADLAASLKLTETQVKIWFQNRRYKTKRRQMAADLLASAPAAKKVAVKVLVRDDQRQYLPGEVLRPPSLLPLQPS

SEQ ID NO: 29 - protein, 282 aa, Homo sapiens
MSRQTATALPTGTSKCPPSQRVPALTGTTASNNDLASLFECPVCFDYVLPPILQCQSGHLVCSNCRPKLTCCPTCRGPLGSIRNLAMEKVANSVLFPCKYASSGCEITLPHTEKADHEELCEFRPYSCPCPGASCKWQGSLDAVMPHLMHQHKSITTLQGEDIVFLATDINLPGAVDWVMMQSCFGFHFMLVLEKQEKYDGHQQFFAIVQLIGTRKQAENFAYRLELNGHRRRLTWEATPRSIHEGIATAIMNSDCLVFDTSIAQLFAENGNLGINVTISMC

SEQ ID NO: 30 - DNA, 1540 bp, Homo sapiens
gtcccgtcggtctcggcgccgggaagaggcggtggcgctgcccgcggtggcgggggttggcgacggagcgcgttggtgccaggaccggggtccgaggcgcgctctccgcccacagaaatgagccgtcagactgctacagcattacctaccggtacctcgaagtgtccaccatcccagagggtgcctgccctgactggcacaactgcatccaacaatgacttggcgagtctttttgagtgtccagtctgctttgactatgtgttaccgcccattcttcaatgtcagagtggccatcttgtttgtagcaactgtcgcccaaagctcacatgttgtccaacttgccggggccctttgggatccattcgcaacttggctatggagaaagtggctaattcagtacttttcccctgtaaatatgcgtcttctggatgtgaaataactctgccacacacagaaaaagcagaccatgaagagctctgtgagtttaggccttattcctgtccgtgccctggtgcttcctgtaaatggcaaggctctctggatgctgtaatgccccatctgatgcatcagcataagtccattacaaccctacagggagaggatatagtttttcttgctacagacattaatcttcctggtgctgttgactgggtgatgatgcagtcctgttttggctttcacttcatgttagtcttagagaaacaggaaaaatacgatggtcaccagcagttcttcgcaatcgtacagctgataggaacacgcaagcaagctgaaaattttgcttaccgacttgagctaaatggtcataggcgacgattgacttgggaagcgactcctcgatctattcatgaaggaattgcaacagccattatgaatagcgactgtctagtctttgacaccagcattgcacagctttttgcagaaaatggcaatttaggcatcaatgtaactatttccatgtgttgaaatggcaatcaaacattttctggccagtgtttaaaacttcagtttcacagaaaataaggcacccatctgtctgccaacctaaaactctttcggtaggtggaagctagacacatgaaggtaaataaaaagaaaggctgttaaatacaggaaacagttgcatgtagtaacactaatatatttaaaaataagtcaacagtaaaccactgaaaaaatatatgtatatacacccaagatgggcatcttttgtattaagaaaggaagcattgtaaaataattctgagttttgtgtttgttgtagattgattgtattgttgaaaaagtttgtttttgcgtgggagtgtgtgcctgcgtgggtgtgtgcgtgtttgggtttttttcctttaactgacaagccatcttgagtggtcatgggccactgcttttccctttgtgagtcaatacatagtgctgctgtgtgctttttttgtgtgtatttgctaatttttattaattttagtttttcattaaataaatttgacttttctgtaaaaaaaaaaaaaaaaaaaaaaaaaaaaaaaaaaaaaaaaaaaaaaaa

SEQ ID NO: 31 - protein, 317 aa, Homo sapiens
MFQAAERPQEWAMEGPRDGLKKERLLDDRHDSGLDSMKDEEYEQMVKELQEIRLEPQEVPRGSEPWKQQLTEDGDSFLHLAIIHEEKALTMEVIRQVKGDLAFLNFQNNLQQTPLHLAVITNQPEIAEALLGAGCDPELRDFRGNTPLHLACEQGCLASVGVLTQSCTTPHLHSILKATNYNGHTCLHLASIHGYLGIVELLVSLGADVNAQEPCNGRTALHLAVDLQNPDLVSLLLKCGADVNRVTYQGYSPYQLTWGRPSTRIQQQLGQLTLENLQMLPESEDEESYDTESEFTEFTEDELPYDDCVFGGQRLTL

SEQ ID NO: 32 - protein, 9 aa, Artificial Sequence
  amino acid sequence of Human influenza hemagglutinin
YPYDVPDYA

SEQ ID NO: 33 - protein, 10 aa, Artificial Sequence
  amino acid sequence of Myc
EQKLISEEDL

SEQ ID NO: 34 - DNA, 10 bp, Artificial Sequence
  amino acid sequence of NF-kappaB specific DNA binding site
gggaatttcc

SEQ ID NO: 35 - protein, 54 aa, Artificial Sequence
  112-165 aa fragment of Nkx3.2
GASGAGLAGGSLSLGQPVCELAASKDLEEEAAGRSDSEMSASVSGDRSPRTEDD

SEQ ID NO: 36 - DNA, 162 bp, Artificial Sequence
  nucleotide sequence encoding 112-165 aa fragment of Nkx3.2
ggggccagcggggccggccttgcggggggatccttgagcctcggccagccggtctgtgagctggccgcttccaaagacctagaggaggaagccgcgggccggagcgacagcgagatgtccgccagcgtctcaggcgaccgcagcccaaggaccgaggacgac

SEQ ID NO: 37 - protein, 164 aa, Artificial Sequence
  154-317 aa fragment of Nkx3.2
VSGDRSPRTEDDGVGPRGAHVSALCSGAGGGGGSGPAGVAEEEEEPAAPKPRKKRSRAAFSHAQVFELERRFNHQRYLSGPERADLAASLKLTETQVKIWFQNRRYKTKRRQMAADLLASAPAAKKVAVKVLVRDDQRQYLPGEVLRPPSLLPLQPSYYYPYYC

SEQ ID NO: 38 - DNA, 492 bp, Artificial Sequence
  nucleotide sequence encoding 154-317 aa fragment of Nkx3.2
gtctcaggcgaccgcagcccaaggaccgaggacgacggtgttggccccagaggtgcacacgtgtccgcgctgtgcagcggggccggcggcgggggcggcagcgggccggcaggcgtcgcggaggaggaggaggagccggcggcgcccaagccacgcaagaagcgctcgcgggccgctttctcccacgcgcaggtcttcgagctggagcgccgctttaaccaccagcgctacctgtccgggcccgagcgcgcagacctggccgcgtcgctgaagctcaccgagacgcaggtgaaaatctggttccagaaccgtcgctacaagacaaagcgccggcagatggcagccgacctgctggcctcggcgcccgccgccaagaaggtggccgtaaaggtgctggtgcgcgacgaccagagacaatacctgcccggcgaagtgctgcggccaccctcgcttctgccactgcagccctcctactattacccgtactactgc

SEQ ID NO: 39 - protein, 42 aa, Artificial Sequence
  112-153 aa fragment of Nkx3.2
GASGAGLAGGSLSLGQPVCELAASKDLEEEAAGRSDSEMSAS

SEQ ID NO: 40 - DNA, 126 bp, Artificial Sequence
  nucleotide sequence encoding 112-153 aa fragment of Nkx3.2
ggggccagcggggccggccttgcggggggatccttgagcctcggccagccggtctgtgagctggccgcttccaaagacctagaggaggaagccgcgggccggagcgacagcgagatgtccgccagc

SEQ ID NO: 41 - protein, 16 aa, Artificial Sequence
  318-333 aa fragment of Nkx3.2
LPGWALSTCAAAAGTQ

SEQ ID NO: 42 - DNA, 48 bp, Artificial Sequence
  nucleotide sequence encoding 318-333 aa fragment of Nkx3.2
ctcccaggctgggcgctctccacctgcgcagctgccgcaggcacccag